European Patent Application EP 4 403 213 A2, published July 24, 2024. Title: METHODS FOR REDUCING CARDIOVASCULAR RISK. Applicant: Sanofi Biotechnology. Application EP. The sequence listing filed with the application follows.

SEQUENCE LISTING (198 sequences)

SEQ ID NO: 1 - protein, 118 aa, synthetic construct [sequence omitted]

SEQ ID NO: 2 - protein, 8 aa, synthetic construct
  REGION 1..8: note = Description of Artificial Sequence: Synthetic peptide
GFTFNNYA

SEQ ID NO: 3 - protein, 8 aa, synthetic construct
  REGION 1..8: note = Description of Artificial Sequence: Synthetic peptide
ISGSGGTT

SEQ ID NO: 4 - protein, 11 aa, synthetic construct
  REGION 1..11: note = Description of Artificial Sequence: Synthetic peptide
AKDSNWGNFDL

SEQ ID NO: 5 - protein, 447 aa, synthetic construct
  REGION 1..447: note = Description of Artificial Sequence: Synthetic REGN727 heavy chain polypeptide
EVQLVESGGGLVQPGGSLRLSCAASGFTFNNYAMNWVRQAPGKGLDWVSTISGSGGTTNYADSVKGRFIISRDSSKHTLYLQMNSLRAEDTAVYYCAKDSNWGNFDLWGRGTLVTVSSASTKGPSVFPLAPSSKSTSGGTAALGCLVKDYFPEPVTVSWNSGALTSGVHTFPAVLQSSGLYSLSSVVTVPSSSLGTQTYICNVNHKPSNTKVDKKVEPKSCDKTHTCPPCPAPELLGGPSVFLFPPKPKDTLMISRTPEVTCVVVDVSHEDPEVKFNWYVDGVEVHNAKTKPREEQYNSTYRVVSVLTVLHQDWLNGKEYKCKVSNKALPAPIEKTISKAKGQPREPQVYTLPPSRDELTKNQVSLTCLVKGFYPSDIAVEWESNGQPENNYKTTPPVLDSDGSFFLYSKLTVDKSRWQQGNVFSCSVMHEALHNHYTQKSLSLSPG

SEQ ID NO: 6 - protein, 113 aa, synthetic construct [sequence omitted]

SEQ ID NO: 7 - protein, 12 aa, synthetic construct
  REGION 1..12: note = Description of Artificial Sequence: Synthetic peptide
QSVLYRSNNRNF

SEQ ID NO: 8 - skipped

SEQ ID NO: 9 - protein, 220 aa, synthetic construct
  REGION 1..220: note = Description of Artificial Sequence: Synthetic REGN727 light chain polypeptide
DIVMTQSPDSLAVSLGERATINCKSSQSVLYRSNNRNFLGWYQQKPGQPPNLLIYWASTRESGVPDRFSGSGSGTDFTLTISSLQAEDVAVYYCQQYYTTPYTFGQGTKLEIKRTVAAPSVFIFPPSDEQLKSGTASVVCLLNNFYPREAKVQWKVDNALQSGNSQESVTEQDSKDSTYSLSSTLTLSKADYEKHKVYACEVTHQGLSSPVTKSFNRGEC

SEQ ID NO: 10 - protein, 9 aa, synthetic construct
  REGION 1..9: note = Description of Artificial Sequence: Synthetic peptide
QQYYTTPYT

SEQ ID NO: 11 - protein, 127 aa, synthetic construct
  REGION 1..127: note = Description of Artificial Sequence: Synthetic polypeptide
EMQLVESGGGLVQPGGSLRLSCAASGFTFSSHWMKWVRQAPGKGLEWVANINQDGSEKYYVDSVKGRFTISRDNAKNSLFLQMNSLRAEDTAVYYCARDIVLMVYDMDYYYYGMDVWGQGTTVTVSS

SEQ ID NO: 12 - protein, 8 aa, synthetic construct
  REGION 1..8: note = Description of Artificial Sequence: Synthetic peptide
GFTFSSHW

SEQ ID NO: 13 - protein, 8 aa, synthetic construct
  REGION 1..8: note = Description of Artificial Sequence: Synthetic peptide
INQDGSEK

SEQ ID NO: 14 - protein, 20 aa, synthetic construct
  REGION 1..20: note = Description of Artificial Sequence: Synthetic peptide
ARDIVLMVYDMDYYYYGMDV

SEQ ID NO: 15 - protein, 112 aa, synthetic construct
  REGION 1..112: note = Description of Artificial Sequence: Synthetic polypeptide
DIVMTQSPLSLPVTPGEPASISCRSSQSLLHSNGNNYLDWYLQKPGQSPQLLIYLGSNRASGVPDRFSGSGSGTDFTLKISRVEAEDVGVYYCMQTLQTPLTFGGGTKVEIK

SEQ ID NO: 16 - protein, 11 aa, synthetic construct
  REGION 1..11: note = Description of Artificial Sequence: Synthetic peptide
QSLLHSNGNNY

SEQ ID NO: 17 - skipped

SEQ ID NO: 18 - protein, 9 aa, synthetic construct
  REGION 1..9: note = Description of Artificial Sequence: Synthetic peptide
MQTLQTPLT

SEQ ID NO: 19 - protein, 8 aa, synthetic construct
  REGION 1..8: note = Description of Artificial Sequence: Synthetic peptide
GFTFSSHW

SEQ ID NO: 20 - protein, 8 aa, synthetic construct
  REGION 1..8: note = Description of Artificial Sequence: Synthetic peptide
INQDGSEK

SEQ ID NO: 21 - protein, 20 aa, synthetic construct
  REGION 1..20: note = Description of Artificial Sequence: Synthetic peptide
ARDIVLMVYDMDYYYYGMDV

SEQ ID NO: 22 - protein, 11 aa, synthetic construct
  REGION 1..11: note = Description of Artificial Sequence: Synthetic peptide
QSLHHSNGNNY

SEQ ID NO: 23 - skipped

SEQ ID NO: 24 - protein, 9 aa, synthetic construct
  REGION 1..9: note = Description of Artificial Sequence: Synthetic peptide
MQTLQTPLT

SEQ ID NO: 25 - protein, 8 aa, synthetic construct
  REGION 1..8: note = Description of Artificial Sequence: Synthetic peptide
GFTFSSHW

SEQ ID NO: 26 - protein, 8 aa, synthetic construct
  REGION 1..8: note = Description of Artificial Sequence: Synthetic peptide
INQDGSEK

SEQ ID NO: 27 - protein, 20 aa, synthetic construct
  REGION 1..20: note = Description of Artificial Sequence: Synthetic peptide
ARDIVLMVYHMDYYYYGMDV

SEQ ID NO: 28 - protein, 11 aa, synthetic construct
  REGION 1..11: note = Description of Artificial Sequence: Synthetic peptide
QSLLHSNGNNY

SEQ ID NO: 29 - skipped

SEQ ID NO: 30 - protein, 9 aa, synthetic construct
  REGION 1..9: note = Description of Artificial Sequence: Synthetic peptide
MQTLQTPLT

SEQ ID NO: 31 - protein, 8 aa, synthetic construct
  REGION 1..8: note = Description of Artificial Sequence: Synthetic peptide
GFTFSSHW

SEQ ID NO: 32 - protein, 8 aa, synthetic construct
  REGION 1..8: note = Description of Artificial Sequence: Synthetic peptide
INQDGSEK

SEQ ID NO: 33 - protein, 20 aa, synthetic construct
  REGION 1..20: note = Description of Artificial Sequence: Synthetic peptide
ARDIVLMVYHMDYYYYGMDV

SEQ ID NO: 34 - protein, 11 aa, synthetic construct
  REGION 1..11: note = Description of Artificial Sequence: Synthetic peptide
QSLHHSNGNNY

SEQ ID NO: 35 - skipped

SEQ ID NO: 36 - protein, 9 aa, synthetic construct
  REGION 1..9: note = Description of Artificial Sequence: Synthetic peptide
MQTLQTPLT

SEQ ID NO: 37 - protein, 131 aa, synthetic construct
  REGION 1..131: note = Description of Artificial Sequence: Synthetic VH; m2CX1D05 polypeptide
QVQLVQSGAEVKKPGSSVKVSCKASGGTFNSHAISWVRQAPGQGLEWMGGINPILGIANYAQKFQGRVTITADESTSTAYMELSSLRSEDTAVYYCARHYEIQIGRYGMNVYYLMYRFASWGQGTLVTVSS

SEQ ID NO: 38 - protein, 10 aa, synthetic construct
  REGION 1..10: note = Description of Artificial Sequence: Synthetic VH CDR1; m2CX1D05 peptide
GGTFNSHAIS

SEQ ID NO: 39 - protein, 20 aa, synthetic construct
  REGION 1..20: note = Description of Artificial Sequence: Synthetic VH CDR2; m2CX1D05 peptide
WMGGINPILGIANYAQKFQG

SEQ ID NO: 40 - protein, 22 aa, synthetic construct
  REGION 1..22: note = Description of Artificial Sequence: Synthetic VH CDR3; m2CX1D05 peptide
HYEIQIGRYGMNVYYLMYRFAS

SEQ ID NO: 41 - protein, 213 aa, synthetic construct
  REGION 1..213: note = Description of Artificial Sequence: Synthetic LC; m2CX1D05 polypeptide
DIQMTQSPSSLSASVGDRVTITCRASQGIRSALNWYQQKPGKAPKLLIYNGSTLQSGVPSRFSGSGSGTDFTLTISSLQPEDFAVYYCQQFDGDPTFGQGTKVEIKRTVAAPSVFIFPPSDEQLKSGTASVVCLLNNFYPREAKVQWKVDNALQSGNSQESVTEQDSKDSTYSLSSTLTLSKADYEKHKVYACEVTHQGLSSPVTKSFNRGEA

SEQ ID NO: 42 - protein, 11 aa, synthetic construct
  REGION 1..11: note = Description of Artificial Sequence: Synthetic VL CDR 1; m2CX1D05 peptide
RASQGIRSALN

SEQ ID NO: 43 - protein, 11 aa, synthetic construct
  REGION 1..11: note = Description of Artificial Sequence: Synthetic VL CDR2; m2CX1D05 peptide
LLIYNGSTLQS

SEQ ID NO: 44 - protein, 7 aa, synthetic construct
  REGION 1..7: note = Description of Artificial Sequence: Synthetic VL CDR3; m2CX1D05 peptide
QQFDGDP

SEQ ID NO: 45 - protein, 119 aa, synthetic construct
  REGION 1..119: note = Description of Artificial Sequence: Synthetic VH; 1B20 polypeptide
QVQLVQSGAEVKKPGESLKISCKGSGYSFTNYWISWVRQMPGKGLEWMGIIYPGDSYTNYSPSFQGQVTISADKSISTAYLQWSSLKASDTAMYYCARDYWYKPLFDIWGQGTLVTVSS

SEQ ID NO: 46 - protein, 10 aa, synthetic construct
  REGION 1..10: note = Description of Artificial Sequence: Synthetic VH CDR1; 1B20 peptide
GYSFTNYWIS

SEQ ID NO: 47 - protein, 20 aa, synthetic construct
  REGION 1..20: note = Description of Artificial Sequence: Synthetic VH CDR2; 1B20 peptide
WMGIIYPGDSYTNYSPSFQG

SEQ ID NO: 48 - protein, 10 aa, synthetic construct
  REGION 1..10: note = Description of Artificial Sequence: Synthetic VH CDR3; 1B20 peptide
DYWYKPLFDI

SEQ ID NO: 49 - protein, 220 aa, synthetic construct
  REGION 1..220: note = Description of Artificial Sequence: Synthetic LC; 1B20 polypeptide
DIVMTQSPDSLAVSLGERATINCRSSQSVLYSSNNKNYLAWYQQKPGQPPKLLIYWASTRESGVPDRFSGSGSGTDFTLTISSLQAEDVAVYYCQQYSSFPITFGQGTKVEIKRTVAAPSVFIFPPSDEQLKSGTASVVCLLNNFYPREAKVQWKVDNALQSGNSQESVTEQDSKDSTYSLSSTLTLSKADYEKHKVYACEVTHQGLSSPVTKSFNRGEA

SEQ ID NO: 50 - protein, 17 aa, synthetic construct
  REGION 1..17: note = Description of Artificial Sequence: Synthetic VL CDR1; 1B20 peptide
RSSQSVLYSSNNKNYLA

SEQ ID NO: 51 - protein, 11 aa, synthetic construct
  REGION 1..11: note = Description of Artificial Sequence: Synthetic VL CDR2; 1B20 peptide
LLIYWASTRES

SEQ ID NO: 52 - protein, 8 aa, synthetic construct
  REGION 1..8: note = Description of Artificial Sequence: Synthetic VL CDR3; 1B20 peptide
QQYSSFPI

SEQ ID NO: 53 - protein, 120 aa, synthetic construct
  REGION 1..120: note = Description of Artificial Sequence: Synthetic variable heavy antibody region polypeptide
EVQLLESGGGLVQPGGSLRLSCKASGYTFSSYGMYWVRQAPGKGLEWIGWIDPGSGGTKYNEKFKGKATISRDNSKNTLYLQMNSLRAEDTAVYYCARERYGYYFDYWGQGTLVTVSSAS

SEQ ID NO: 54 - protein, 16 aa, synthetic construct
  REGION 1..16: note = Description of Artificial Sequence: Synthetic AX132 heavy chain CDR1 antibody region peptide
KASGYTFSSYGMYWVR

SEQ ID NO: 55 - protein, 23 aa, synthetic construct
  REGION 1..23: note = Description of Artificial Sequence: Synthetic AX132 heavy chain CDR2 antibody region peptide
WIGWIDPGSGGTKYNEKFKGKAT

SEQ ID NO: 56 - protein, 15 aa, synthetic construct
  REGION 1..15: note = Description of Artificial Sequence: Synthetic AX132 heavy chain CDR3 antibody region peptide
CARERYGYYFDYWGQ

SEQ ID NO: 57 - protein, 108 aa, synthetic construct
  REGION 1..108: note = Description of Artificial Sequence: Synthetic variable light antibody region polypeptide
EIVLTQSPATLSLSPGERATITCRASQYVGSYLNWYQQKPGQAPRLLIYDASNRATGIPARFSGSGSGTDFTLTISSLEPEDFAVYYCQVWDSSPPVVFGGGTKVEIK

SEQ ID NO: 58 - protein, 17 aa, synthetic construct
  REGION 1..17: note = Description of Artificial Sequence: Synthetic AX213 and AX132 light chain CDR1 antibody region peptide
ITCRASQYVGSYLNWYQ

SEQ ID NO: 59 - protein, 13 aa, synthetic construct
  REGION 1..13: note = Description of Artificial Sequence: Synthetic AX213 and AX132 light chain CDR2 antibody region peptide
LIYDASNRATGIP

SEQ ID NO: 60 - protein, 16 aa, synthetic construct
  REGION 1..16: note = Description of Artificial Sequence: Synthetic AX132 & AX213 light chain CDR3 antibody region peptide
YYCQVWDSSPPVVFGG

SEQ ID NO: 61 - protein, 120 aa, synthetic construct
  REGION 1..120: note = Description of Artificial Sequence: Synthetic variable heavy antibody region polypeptide
EVQLLESGGGLVQPGGSLRLSCKASGYTFSRYGINWVRQAPGKGLEWIGRIDPGNGGTRYNEKFKGKATISRDNSKNTLYLQMNSLRAEDTAVYYCARANDGYSFDYWGQGTLVTVSSAS

SEQ ID NO: 62 - protein, 16 aa, synthetic construct
  REGION 1..16: note = Description of Artificial Sequence: Synthetic AX213 heavy chain CDR1 antibody region peptide
KASGYTFSRYGINWVR

SEQ ID NO: 63 - protein, 23 aa, synthetic construct
  REGION 1..23: note = Description of Artificial Sequence: Synthetic AX213 heavy chain CDR2 antibody region peptide
WIGRIDPGNGGTRYNEKFKGKAT

SEQ ID NO: 64 - protein, 15 aa, synthetic construct
  REGION 1..15: note = Description of Artificial Sequence: Synthetic AX213 heavy chain CDR3 antibody region peptide
CARANDGYSFDYWGQ

SEQ ID NO: 65 - protein, 108 aa, synthetic construct; identical to SEQ ID NO: 57
  REGION 1..108: note = Description of Artificial Sequence: Synthetic variable light antibody region polypeptide

SEQ ID NO: 66 - protein, 17 aa, synthetic construct
  REGION 1..17: note = Description of Artificial Sequence: Synthetic AX213 and AX132 light chain CDR1 antibody region peptide
ITCRASQYVGSYLNWYQ

SEQ ID NO: 67 - protein, 13 aa, synthetic construct
  REGION 1..13: note = Description of Artificial Sequence: Synthetic AX213 and AX132 light chain CDR2 antibody region peptide
LIYDASNRATGIP

SEQ ID NO: 68 - protein, 16 aa, synthetic construct
  REGION 1..16: note = Description of Artificial Sequence: Synthetic AX132 & AX213 light chain CDR3 antibody region peptide
YYCQVWDSSPPVVFGG

SEQ ID NO: 69 - protein, 119 aa, synthetic construct
  REGION 1..119: note = Description of Artificial Sequence: Synthetic AX1 VH antibody sequence polypeptide
EVQLLESGGGLVQPGGSLRLSCKASGFTFTSYYMHWVRQAPGKGLEWIGRINPDSGSTKYNEKFKGRATISRDNSKNTLYLQMNSLRAEDTAVYYCARGGRLSWDFDVWGQGTLVTVSS

SEQ ID NO: 70 - protein, 16 aa, synthetic construct
  REGION 1..16: note = Description of Artificial Sequence: Synthetic AX1 VH CDR1 antibody sequence peptide
KASGFTFTSYYMHWVR

SEQ ID NO: 71 - protein, 23 aa, synthetic construct
  REGION 1..23: note = Description of Artificial Sequence: Synthetic AX1 VH CDR2 antibody sequence peptide
WIGRINPDSGSTKYNEKFKGRAT

SEQ ID NO: 72 - protein, 16 aa, synthetic construct
  REGION 1..16: note = Description of Artificial Sequence: Synthetic AX1 VH CDR3 antibody sequence peptide
CARGGRLSWDFDVWGQ

SEQ ID NO: 73 - protein, 109 aa, synthetic construct
  REGION 1..109: note = Description of Artificial Sequence: Synthetic AX1 VL antibody sequence polypeptide
DIQMTQSPSSLSASVGDRVTITCRASQDISRYLAWYQQKPGKAPKLLIYAASSLQSGVPSRFSGSGSGTDFTLTISSLQPEDFATYYCAAYDYSLGGYVFGDGTKVEIK

SEQ ID NO: 74 - protein, 11 aa, synthetic construct
  REGION 1..11: note = Description of Artificial Sequence: Synthetic AX1 VL CDR1 antibody sequence peptide
RASQDISRYLA

SEQ ID NO: 75 - protein, 7 aa, synthetic construct
  REGION 1..7: note = Description of Artificial Sequence: Synthetic AX1 AX9 AX189 VL CDR2 antibody sequence peptide
AASSLQS

SEQ ID NO: 76 - protein, 11 aa, synthetic construct
  REGION 1..11: note = Description of Artificial Sequence: Synthetic AX1 VL CDR3 antibody sequence peptide
AAYDYSLGGYV

SEQ ID NO: 77 - protein, 121 aa, synthetic construct
  REGION 1..121: note = Description of Artificial Sequence: Synthetic AX9 AX189 VH antibody sequence polypeptide
EVQLLESGGGLVQPGGSLRLSCKASGYTFSSYWMHWVRQAPGKGLEWIGRIDPYNGGTKYNEKFKGKATISRDNSKNTLYLQMNSLRAEDTAVYYCARYGYYLGSYAMDYWGQGTLVTVSS

SEQ ID NO: 78 - protein, 16 aa, synthetic construct
  REGION 1..16: note = Description of Artificial Sequence: Synthetic AX9 AX189 VH CDR1 antibody sequence peptide
KASGYTFSSYWMHWVR

SEQ ID NO: 79 - protein, 23 aa, synthetic construct
  REGION 1..23: note = Description of Artificial Sequence: Synthetic AX9 AX189 VH CDR2 antibody sequence peptide
WIGRIDPYNGGTKYNEKFKGKAT

SEQ ID NO: 80 - protein, 18 aa, synthetic construct
  REGION 1..18: note = Description of Artificial Sequence: Synthetic AX9 AX189 VH CDR3 antibody sequence peptide
CARYGYYLGSYAMDYWGQ

SEQ ID NO: 81 - protein, 109 aa, synthetic construct
  REGION 1..109: note = Description of Artificial Sequence: Synthetic AX189 VL antibody sequence polypeptide
DIQMTQSPSSLSASVGDRVTITCRASQDVSRYLTWYQQKPGKAPKLLIYAASSLQSGVPSRFSGSGSGTDFTLTISSLQPEDFATYYCQAYDYSLSGYVFGGGTKVEIK

SEQ ID NO: 82 - protein, 11 aa, synthetic construct
  REGION 1..11: note = Description of Artificial Sequence: Synthetic AX189 VL CDR1 antibody sequence peptide
RASQDVSRYLT

SEQ ID NO: 83 - protein, 7 aa, synthetic construct
  REGION 1..7: note = Description of Artificial Sequence: Synthetic AX1 AX9 AX189 VL CDR2 antibody sequence peptide
AASSLQS

SEQ ID NO: 84 - protein, 11 aa, synthetic construct
  REGION 1..11: note = Description of Artificial Sequence: Synthetic AX189 VL CDR3 antibody sequence peptide
QAYDYSLSGYV

SEQ ID NO: 85 - protein, 115 aa, Homo sapiens
QVQLVQSGAEVKKPGASVKVSCKASGYTLTSYGISWVRQAPGQGLEWMGWVSFYNGNTNYAQKLQGRGTMTTDPSTSTAYMELRSLRSDDTAVYYCARGYGMDVWGQGTTVTVSS

SEQ ID NO: 86 - protein, 5 aa, Homo sapiens
SYGIS

SEQ ID NO: 87 - protein, 17 aa, Homo sapiens
WVSFYNGNTNYAQKLQG

SEQ ID NO: 88 - protein, 6 aa, Homo sapiens
GYGMDV

SEQ ID NO: 89 - protein, 109 aa, Homo sapiens
QSALTQPASVSGSPGQSITISCTGTSSDVGGYNSVSWYQQHPGKAPKLMIYEVSNRPSGVSNRFSGSKSGNTASLTISGLQAEDEADYYCNSYTSTSMVFGGGTKLTVL

SEQ ID NO: 90 - protein, 14 aa, Homo sapiens
TGTSSDVGGYNSVS

SEQ ID NO: 91 - protein, 7 aa, Homo sapiens
EVSNRPS

SEQ ID NO: 92 - protein, 9 aa, Homo sapiens
NSYTSTSMV

SEQ ID NO: 93 - protein, 123 aa, Homo sapiens
EVQLVESGGGLVKPGGSLRLSCAASGFTFSSYSMNWVRQAPGKGLEWVSSISSSSSYISYADSVKGRFTISRDNAKNSLYLQMNSLRAEDTAVYFCARDYDFWSAYYDAFDVWGQGTMVTVSS

SEQ ID NO: 94 - protein, 10 aa, Homo sapiens
GFTFSSYSMN

SEQ ID NO: 95 - protein, 17 aa, Homo sapiens
SISSSSSYISYADSVKG

SEQ ID NO: 96 - protein, 14 aa, Homo sapiens
DYDFWSAYYDAFDV

SEQ ID NO: 97 - protein, 111 aa, Homo sapiens
QSVLTQPPSVSGAPGQRVTISCTGSSSNIGAGYDVHWYQQLPGTAPKLLISGNSNRPSGVPDRFSGSKSGTSASLAITGLQAEDEADYYCQSYDSSLSGSVFGGGTKLTVL

SEQ ID NO: 98 - protein, 14 aa, Homo sapiens
TGSSSNIGAGYDVH

SEQ ID NO: 99 - protein, 7 aa, Homo sapiens
GNSNRPS

SEQ ID NO: 100 - protein, 11 aa, Homo sapiens
QSYDSSLSGSV

SEQ ID NO: 101 - protein, 114 aa, Homo sapiens
QVQLVESGGGVAQPGRSLRLSCAASGFTFSSYGMHWVRQAPGKGLEWVAVIYYDGINKHYADSVKGRFTISRDNSKNTLYLQMNSLRAEDTAVYYCARDRGLDWGQGTLVTVSS

SEQ ID NO: 102 - protein, 10 aa, Homo sapiens
GFTFSSYGMH

SEQ ID NO: 103 - protein, 17 aa, Homo sapiens
VIYYDGINKHYADSVKG

SEQ ID NO: 104 - protein, 5 aa, Homo sapiens
DRGLD

SEQ ID NO: 105 - protein, 113 aa, Homo sapiens
DIVMTQSPDSLAVSLGERATINCKSSQSVLYSSNSKNYLVWYQQKPGQPPKLLIYWASTRESGVPDRFSGSGSGTDFTLTISSLQAEDVAVYYCQQYYSTPWTFGQGTKVEIK

SEQ ID NO: 106 - protein, 17 aa, Homo sapiens
KSSQSVLYSSNSKNYLV

SEQ ID NO: 107 - protein, 7 aa, Homo sapiens
WASTRES

SEQ ID NO: 108 - protein, 9 aa, Homo sapiens
QQYYSTPWT

SEQ ID NO: 109 - protein, 118 aa, synthetic construct
  REGION 1..118: note = Description of Artificial Sequence: Synthetic anti-PCSK9 monoclonal antibody pJG04 (clones LGT-209 and LGT-210) Vh heavy chain variable region (FR1-FR4) polypeptide
QVQLVQSGAEVKKPGASVKVSCKASGYTFSTMYMSWVRQAPGQGLEWMGRIDPANEHTNYAQKFQGRVTMTRDTSISTAYMELSRLTSDDTAVYYCARSYYYYNMDYWGQGTLVTVSS

SEQ ID NO: 110 - protein, 5 aa, synthetic construct
  REGION 1..5: note = Description of Artificial Sequence: Synthetic anti-PCSK9 monoclonal antibody clones LGT-209, LGT-210 and LGT-211 heavy chain CDR1 peptide
TMYMS

SEQ ID NO: 111 - protein, 17 aa, synthetic construct
  REGION 1..17: note = Description of Artificial Sequence: Synthetic anti-PCSK9 monoclonal antibody clones LGT-209, LGT-210 and LGT-211 heavy chain CDR2 peptide
RIDPANEHTNYAQKFQG

SEQ ID NO: 112 - protein, 9 aa, synthetic construct
  REGION 1..9: note = Description of Artificial Sequence: Synthetic anti-PCSK9 monoclonal antibody pJG04(clones LGT-209 and LGT-210) Vh heavy chain complementarity determining region 3 (CDR3) peptide
SYYYYNMDY

SEQ ID NO: 113 - protein, 106 aa, synthetic construct
  REGION 1..106: note = Description of Artificial Sequence: Synthetic anti-PCSK9 monoclonal antibody pJG10(clones LGT-209 and LGT-211) Vk light chain variable region (FR1-FR4) polypeptide
QIVLTQSPATLSVSPGERATLSCRASQSVSYMHWYQQKPGQAPRLLIYGVFRRATGIPDRFSGSGSGTDFTLTIGRLEPEDFAVYYCLQWSSDPPTFGQGTKLEIK

SEQ ID NO: 114 - protein, 10 aa, synthetic construct
  REGION 1..10: note = Description of Artificial Sequence: Synthetic anti-PCSK9 monoclonal antibody clones LGT-209, LGT-210 and LGT-211 light chain CDR1 peptide
RASQSVSYMH

SEQ ID NO: 115 - protein, 7 aa, synthetic construct
  REGION 1..7: note = Description of Artificial Sequence: Synthetic anti-PCSK9 monoclonal antibody clones LGT-209, LGT-210 and LGT-211 light chain CDR1 peptide
GVFRRAT

SEQ ID NO: 116 - protein, 9 aa, synthetic construct
  REGION 1..9: note = Description of Artificial Sequence: Synthetic mouse anti-PCSK9 monoclonal antibody LFU720 and anti-PCSK9 monoclonal antibody clones LGT-209, LGT-210 and LGT-211 light chain CDR3 peptide
LQWSSDPPT

SEQ ID NO: 117 - protein, 118 aa, Homo sapiens
QVQLVQSGAEVKKPGASVKVSCKASGYTFTSYYMHWVRQAPGQGLEWMGEISPFGGRTNYNEKFKSRVTMTRDTSTSTVYMELSSLRSEDTAVYYCARERPLYASDLWGQGTTVTVSS

SEQ ID NO: 118 - protein, 7 aa, synthetic construct
  REGION 1..7: note = Description of Artificial Sequence: Synthetic peptide
GYTFTSY

SEQ ID NO: 119 - protein, 6 aa, synthetic construct
  REGION 1..6: note = Description of Artificial Sequence: Synthetic peptide
SPFGGR

SEQ ID NO: 120 - protein, 9 aa, synthetic construct
  REGION 1..9: note = Description of Artificial Sequence: Synthetic variable heavy chain CDR peptide
ERPLYASDL

SEQ ID NO: 121 - protein, 107 aa, Homo sapiens
DIQMTQSPSSLSASVGDRVTITCRASQGISSALAWYQQKPGKAPKLLIYSASYRYTGVPSRFSGSGSGTDFTFTISSLQPEDIATYYCQQRYSLWRTFGQGTKLEIK

SEQ ID NO: 122 - protein, 11 aa, synthetic construct
  REGION 1..11: note = Description of Artificial Sequence: Synthetic variable light chain CDR peptide
RASQGISSALA

SEQ ID NO: 123 - protein, 7 aa, synthetic construct
  REGION 1..7: note = Description of Artificial Sequence: Synthetic variable light chain CDR peptide
SASYRYT

SEQ ID NO: 124 - protein, 9 aa, synthetic construct
  REGION 1..9: note = Description of Artificial Sequence: Synthetic variable light chain CDR peptide
QQRYSLWRT

SEQ ID NO: 125 - protein, 118 aa, Homo sapiens
QVQLVQSGAEVKKPGASVKVSCKASGYTFTSYYMHWVRQAPGQGLEWMGEIHPSGGRTNYNEKFKSRVTMTRDTSTSTVYMELSSLRSEDTAVYYCARERPLYAMDYWGQGTTVTVSS

SEQ ID NO: 126 - protein, 10 aa, Homo sapiens
GYTFTSYYMH

SEQ ID NO: 127 - protein, 17 aa, Homo sapiens
EIHPSGGRTNYNEKFKS

SEQ ID NO: 128 - protein, 9 aa, Homo sapiens
ERPLYAMDY

SEQ ID NO: 129 - protein, 107 aa, Homo sapiens [sequence omitted]

SEQ ID NO: 130 - protein, 11 aa, Homo sapiens
KASQDVHTAVA

SEQ ID NO: 131 - protein, 7 aa, Homo sapiens
HASYRYT

SEQ ID NO: 132 - protein, 9 aa, Homo sapiens
QQRYSLWRT

SEQ ID NO: 133 - protein, 118 aa, Homo sapiens [sequence omitted]

SEQ ID NO: 134 - protein, 10 aa, Homo sapiens
GYTFTSYYMH

SEQ ID NO: 135 - protein, 17 aa, Homo sapiens
EIHPSGGRTNYNEKFKS

SEQ ID NO: 136 - protein, 9 aa, Homo sapiens
ERPLYASDL

SEQ ID NO: 137 - protein, 107 aa, Homo sapiens [sequence omitted]

SEQ ID NO: 138 - protein, 11 aa, Homo sapiens
KASQDVHTAVA

SEQ ID NO: 139 - protein, 7 aa, Homo sapiens
HASYRYT

SEQ ID NO: 140 - protein, 9 aa, Homo sapiens
QQRYSLWRT

SEQ ID NO: 141 - protein, 118 aa, Mus musculus
QVQLQQPGAELVKPGASVKLSCKASGYTFTSYWMHWVKQRPGQGLEWIGEINPSNGRTNYNEKFKSKATLTVDKSSSTAYMQLSSLTSEDSAVYYCARERPLYAMDYWGQGTSVTVSS

SEQ ID NO: 142 - protein, 7 aa, Mus musculus
GYTFTSY

SEQ ID NO: 143 - protein, 6 aa, Mus musculus
NPSNGR

SEQ ID NO: 144 - protein, 9 aa, Mus musculus
ERPLYAMDY

SEQ ID NO: 145 - protein, 108 aa, Mus musculus
DIVMTQSHKFMSTSVGDRVSITCKASQDVSTAVAWYQQKPGQSPKLLIYSASYRYTGVPDRFTGSGSGTDFTFTISSVQAEDLAVYYCQQRYSTPRTFGGGTKLEIKR

SEQ ID NO: 146 - protein, 11 aa, Mus musculus
KASQDVSTAVA

SEQ ID NO: 147 - protein, 7 aa, synthetic construct
  REGION 1..7: note = Description of Artificial Sequence: Synthetic variable light chain CDR peptide
SASYRYT

SEQ ID NO: 148 - protein, 9 aa, Mus musculus
QQRYSTPRT

SEQ ID NO: 149 - protein, 115 aa, Mus musculus
EVQLQQSGPELVKPGASVKISCKASGYTFTDYYMNWVKQSHGKSLEWIGDINPNNGGTTYNQKFKGKATLTVDKSYSTAYMELRSLTSEDSAVYYCARWLLFAYWGQGTLVTVSA

SEQ ID NO: 150 - protein, 7 aa, Mus musculus
GYTFTDY

SEQ ID NO: 151 - protein, 6 aa, Mus musculus
NPNNGG

SEQ ID NO: 152 - protein, 6 aa, Mus musculus
WLLFAY

SEQ ID NO: 153 - protein, 108 aa, Mus musculus
DIVMTQSQKFMSTSVGDRVSVTCKASQNVGTNVAWYQQKPGQSPKALIYSASYRYSGVPDRFTGSGSGTDFTLTISNVLSEDLAEYFCQQFYSYPYTFGGGTKLEIKR

SEQ ID NO: 154 - protein, 11 aa, Mus musculus
KASQNVGTNVA

SEQ ID NO: 155 - protein, 7 aa, Mus musculus
SASYRYS

SEQ ID NO: 156 - protein, 9 aa, Mus musculus
QQFYSYPYT

SEQ ID NO: 157 - protein, 123 aa, Mus musculus
EVQLQQSGPELVKPGASVKISCKASGYTFTDYYMNWVKQSHGKSLEWIGDINPNNGGTSYNQKFKGKATLTVDKSSSTAYMELRSLTSEDSAVYYCAGGGIYYRYDRNYFDYWGQGTTLTVSS

SEQ ID NO: 158 - protein, 7 aa, Mus musculus
GYTFTDY

SEQ ID NO: 159 - protein, 6 aa, Mus musculus
NPNNGG

SEQ ID NO: 160 - protein, 14 aa, Mus musculus
GGIYYRYDRNYFDY

SEQ ID NO: 161 - protein, 107 aa, Mus musculus
DIQMTQTTSSLSASLGDRVTISCSASQGISNYLNWYQQKPDGTVKLLIYYTSSLHSGVPSRFSGSGSGTDYSLTISNLEPEDIATYYCQQYSKLPFTFGSGTKLEIK

SEQ ID NO: 162 - protein, 11 aa, Mus musculus
SASQGISNYLN

SEQ ID NO: 163 - protein, 7 aa, Mus musculus
YTSSLHS

SEQ ID NO: 164 - protein, 9 aa, synthetic construct
  REGION 1..9: note = Description of Artificial Sequence: Synthetic peptide
QQYSKLPFT

SEQ ID NO: 165 - protein, 117 aa, Mus musculus
EVKLVESEGGLVQPGSSMKLSCTASGFTFSDYYMAWVRQVPEKGLEWVANINYDGSNTSYLDSLKSRFIISRDNAKNILYLQMSSLKSEDTATYYCAREKFAAMDYWGQGTSVTVSS

SEQ ID NO: 166 - protein, 7 aa, Mus musculus
GFTFSDY

SEQ ID NO: 167 - protein, 6 aa, Mus musculus
NYDGSN

SEQ ID NO: 168 - protein, 8 aa, Mus musculus
EKFAAMDY

SEQ ID NO: 169 - protein, 108 aa, Mus musculus
DIVMTQSHKFMSTSFGDRVSITCKASQDVSNALAWYQQKPGHSPKLLIFSASYRYTGVPDRFTGSGSGTDFTFTISSVQAEDLAVYYCQQHYSTPWTFGGGTKLEIKR

SEQ ID NO: 170 - protein, 11 aa, Mus musculus
KASQDVSNALA

SEQ ID NO: 171 - protein, 7 aa, synthetic construct
  REGION 1..7: note = Description of Artificial Sequence: Synthetic variable light chain CDR peptide
SASYRYT

SEQ ID NO: 172 - protein, 9 aa, Mus musculus
QQHYSTPWT

SEQ ID NO: 173 - protein, 121 aa, synthetic construct
  REGION 1..121: note = Description of Artificial Sequence: Synthetic polypeptide
EVQLVESGGGLVQPGGSLRLSCAASGFTFTRHTIHWVRQAPGKGLEWVARISPANGNTNYADSVKGRFTISADTSKNTAYLQMNSLRAEDTAVYYCARWIGSRELYIMDYWGQGTLVTVSS

SEQ ID NO: 174 - protein, 10 aa, synthetic construct
  REGION 1..10: note = Description of Artificial Sequence: Synthetic peptide
GFTFTRHTIH

SEQ ID NO: 175 - protein, 17 aa, synthetic construct
  REGION 1..17: note = Description of Artificial Sequence: Synthetic peptide
RISPANGNTNYADSVKG

SEQ ID NO: 176 - protein, 12 aa, synthetic construct
  REGION 1..12: note = Description of Artificial Sequence: Synthetic peptide
WIGSRELYIMDY

SEQ ID NO: 177 - protein, 108 aa, synthetic construct
  REGION 1..108: note = Description of Artificial Sequence: Synthetic polypeptide
DIQMTQSPSSLSASVGDRVTITCRASQDVSTAVAWYQQKPGKAPKLLIYSASFLYSGVPSRFSGSGSGTDFTLTISSLQPEDFATYYCQQSYRIQPTFGQGTKVEIKR

SEQ ID NO: 178 - protein, 11 aa, synthetic construct
  REGION 1..11: note = Description of Artificial Sequence: Synthetic peptide
RASQDVSTAVA

SEQ ID NO: 179 - protein, 7 aa, synthetic construct
  REGION 1..7: note = Description of Artificial Sequence: Synthetic peptide
SASFLYS

SEQ ID NO: 180 - protein, 9 aa, synthetic construct
  REGION 1..9: note = Description of Artificial Sequence: Synthetic peptide
QQSYRIQPT

SEQ ID NO: 181 - protein, 121 aa, synthetic construct
  REGION 1..121: note = Description of Artificial Sequence: Synthetic polypeptide
EVQLVESGGGLVQPGGSLRLSCAASGFTFSSTAIHWVRQAPGKGLEWVARISPANGNTNYADSVKGRFTISADTSKNTAYLQMNSLRAEDTAVYYCARWIGSRELYIMDYWGQGTLVTVSS

SEQ ID NO: 182 - protein, 10 aa, synthetic construct
  REGION 1..10: note = Description of Artificial Sequence: Synthetic peptide
GFTFSSTAIH

SEQ ID NO: 183 - protein, 17 aa, synthetic construct
  REGION 1..17: note = Description of Artificial Sequence: Synthetic peptide
RISPANGNTNYADSVKG

SEQ ID NO: 184 - protein, 12 aa, synthetic construct
  REGION 1..12: note = Description of Artificial Sequence: Synthetic peptide
WIGSRELYIMDY

SEQ ID NO: 185 - protein, 108 aa, synthetic construct
  REGION 1..108: note = Description of Artificial Sequence: Synthetic polypeptide
DIQMTQSPSSLSASVGDRVTITCRASQDVSTAVAWYQQKPGKAPKLLIYSASFLYSGVPSRFSGSGSGTDFTLTISSLQPEDFATYYCQQSYPALHTFGQGTKVEIKR

SEQ ID NO: 186 - protein, 11 aa, synthetic construct
  REGION 1..11: note = Description of Artificial Sequence: Synthetic peptide
RASQDVSTAVA

SEQ ID NO: 187 - protein, 7 aa, synthetic construct
  REGION 1..7: note = Description of Artificial Sequence: Synthetic peptide
SASFLYS

SEQ ID NO: 188 - protein, 9 aa, synthetic construct
  REGION 1..9: note = Description of Artificial Sequence: Synthetic peptide
QQSYPALHT

SEQ ID NO: 189 - protein, 125 aa, synthetic construct
  REGION 1..125: note = Description of Artificial Sequence: Synthetic polypeptide
EVQLVESGGGLVKPGGSLRLSCAASGFPFSKLGMVWVRQAPGKGLEWVSTISSGGGYTYYPDSVKGRFTISRDNAKNSLYLQMNSLRAEDTAVYYCAREGISFQGGTYTYVMDYWGQGTLVTVSS

SEQ ID NO: 190 - protein, 10 aa, synthetic construct
  REGION 1..10: note = Description of Artificial Sequence: Synthetic peptide
GFPFSKLGMV

SEQ ID NO: 191 - protein, 17 aa, synthetic construct
  REGION 1..17: note = Description of Artificial Sequence: Synthetic peptide
TISSGGGYTYYPDSVKG

SEQ ID NO: 192 - protein, 16 aa, synthetic construct
  REGION 1..16: note = Description of Artificial Sequence: Synthetic peptide
EGISFQGGTYTYVMDY

SEQ ID NO: 193 - protein, 112 aa, synthetic construct
  REGION 1..112: note = Description of Artificial Sequence: Synthetic polypeptide
DIVMTQSPLSLPVTPGEPASISCRSSKSLLHRNGITYSYWYLQKPGQSPQLLIYQLSNLASGVPDRFSGSGSGTDFTLKISRVEAEDVGVYYCYQNLELPLTFGQGTKVEIK

SEQ ID NO: 194 - protein, 16 aa, synthetic construct
  REGION 1..16: note = Description of Artificial Sequence: Synthetic peptide
RSSKSLLHRNGITYSY

SEQ ID NO: 195 - protein, 7 aa, synthetic construct
  REGION 1..7: note = Description of Artificial Sequence: Synthetic peptide
QLSNLAS

SEQ ID NO: 196 - protein, 9 aa, synthetic construct
  REGION 1..9: note = Description of Artificial Sequence: Synthetic peptide
YQNLELPLT

SEQ ID NO: 197 - DNA, 2076 bp, Homo sapiens
  source 1..2076: mol_type = genomic DNA
atgggcaccgtcagctccaggcggtcctggtggccgctgccactgctgctgctgctgctgctgctcctgggtcccgcgggcgcccgtgcgcaggaggacgaggacggcgactacgaggagctggtgctagccttgcgttccgaggaggacggcctggccgaagcacccgagcacggaaccacagccaccttccaccgctgcgccaaggatccgtggaggttgcctggcacctacgtggtggtgctgaaggaggagacccacctctcgcagtcagagcgcactgcccgccgcctgcaggcccaggctgcccgccggggatacctcaccaagatcctgcatgtcttccatggccttcttcctggcttcctggtgaagatgagtggcgacctgctggagctggccttgaagttgccccatgtcgactacatcgaggaggactcctctgtctttgcccagagcatcccgtggaacctggagcggattacccctccacggtaccgggcggatgaataccagccccccgacggaggcagcctggtggaggtgtatctcctagacaccagcatacagagtgaccaccgggaaatcgagggcagggtcatggtcaccgacttcgagaatgtgcccgaggaggacgggacccgcttccacagacaggccagcaagtgtgacagtcatggcacccacctggcaggggtggtcagcggccgggatgccggcgtggccaagggtgccagcatgcgcagcctgcgcgtgctcaactgccaagggaagggcacggttagcggcaccctcataggcctggagtttattcggaaaagccagctggtccagcctgtggggccactggtggtgctgctgcccctggcgggtgggtacagccgcgtcctcaacgccgcctgccagcgcctggcgagggctggggtcgtgctggtcaccgctgccggcaacttccgggacgatgcctgcctctactccccagcctcagctcccgaggtcatcacagttggggccaccaatgcccaagaccagccggtgaccctggggactttggggaccaactttggccgctgtgtggacctctttgccccaggggaggacatcattggtgcctccagcgactgcagcacctgctttgtgtcacagagtgggacatcacaggctgctgcccacgtggctggcattgcagccatgatgctgtctgccgagccggagctcaccctggccgagttgaggcagagactgatccacttctctgccaaagatgtcatcaatgaggcctggttccctgaggaccagcgggtactgacccccaacctggtggccgccctgccccccagcacccatggggcaggttggcagctgttttgcaggactgtatggtcagcacactcggggcctacacggatggccacagccgtcgcccgctgcgccccagatgaggagctgctgagctgctccagtttctccaggagtgggaagcggcggggcgagcgcatggaggcccaagggggcaagctggtctgccgggcccacaacgcttttgggggtgagggtgtctacgccattgccaggtgctgcctgctaccccaggccaactgcagcgtccacacagctccaccagctgaggccagcatggggacccgtgtccactgccaccaacagggccacgtcctcacaggctgcagctcccactgggaggtggaggaccttggcacccacaagccgcctgtgctgaggccacgaggtcagcccaaccagtgcgtgggccacagggaggccagcatccacgcttcctgctgccatgccccaggtctggaatgcaaagtcaaggagcatggaatcccggcccctcaggagcaggtgaccgtggcctgcgaggagggctggaccctgactggctgcagtgccctccctgggacctcccacgtcctgggggcctacgccgtagacaacacgtgtgtagtcaggagccgggacgtcagcactacaggcagcaccagcgaaggggccgtgacagccgttgccatctgctgccggagccggcacctggcgcaggcctcccaggagctccag

SEQ ID NO: 198 - protein, 692 aa, Homo sapiens
MGTVSSRRSWWPLPLLLLLLLLLGPAGARAQEDEDGDYEELVLALRSEEDGLAEAPEHGTTATFHRCAKDPWRLPGTYVVVLKEETHLSQSERTARRLQAQAARRGYLTKILHVFHGLLPGFLVKMSGDLLELALKLPHVDYIEEDSSVFAQSIPWNLERITPPRYRADEYQPPDGGSLVEVYLLDTSIQSDHREIEGRVMVTDFENVPEEDGTRFHRQASKCDSHGTHLAGVVSGRDAGVAKGASMRSLRVLNCQGKGTVSGTLIGLEFIRKSQLVQPVGPLVVLLPLAGGYSRVLNAACQRLARAGVVLVTAAGNFRDDACLYSPASAPEVITVGATNAQDQPVTLGTLGTNFGRCVDLFAPGEDIIGASSDCSTCFVSQSGTSQAAAHVAGIAAMMLSAEPELTLAELRQRLIHFSAKDVINEAWFPEDQRVLTPNLVAALPPSTHGAGWQLFCRTVWSAHSGPTRMATAVARCAPDEELLSCSSFSRSGKRRGERMEAQGGKLVCRAHNAFGGEGVYAIARCCLLPQANCSVHTAPPAEASMGTRVHCHQQGHVLTGCSSHWEVEDLGTHKPPVLRPRGQPNQCVGHREASIHASCCHAPGLECKVKEHGIPAPQEQVTVACEEGWTLTGCSALPGTSHVLGAYAVDNTCVVRSRDVSTTGSTSEGAVTAVAICCRSRHLAQASQELQ